European Patent Specification EP 4 011 363 B1, published October 30, 2024. Title: MINERAL-COATED MICROSPHERES. Applicant: Murphy, Willaim Jongpaiboonkit, Leenaporn. Application PCT/US09/58419. The sequence listing filed with the application follows.

SEQUENCE LISTING (7 sequences)

SEQ ID NO: 1 - protein, 13 aa, Artificial Sequence
  modified peptide derived from osteocalcin
AAAAEPRREVAEL

SEQ ID NO: 2 - protein, 13 aa, Artificial Sequence
  modified peptide derived from osteocalcin
  MISC_FEATURE (5)..(5): carboxyglutamate
  MISC_FEATURE (9)..(9): carboxyglutamate
  MISC_FEATURE (12)..(12): carboxyglutamate
AAAAXPRRXVAXL

SEQ ID NO: 3 - protein, 7 aa, Artificial Sequence
  a cell adhesion peptide derived from fibronectin
GGRGDSP

SEQ ID NO: 4 - protein, 7 aa, Artificial Sequence
  a cell adhesion peptide derived from laminin
GGIKVAV

SEQ ID NO: 5 - protein, 7 aa, Artificial Sequence
  a cell adhesion peptide derived from laminin
GGYIGSR

SEQ ID NO: 6 - protein, 6 aa, Artificial Sequence
  a cell adhesion/signaling peptide derived from type I collagen
GGDGEA

SEQ ID NO: 7 - protein, 22 aa, Artificial Sequence
  a peptide derived from bone morphogenetic protein-2
GGKIPKASSVPTELSAISTLYL